European Patent Specification EP 3 650 543 B1, published June 7, 2023. Title: PC-25879. Applicant: Japan Science and Technology Agency. The sequence listing filed with the application follows.

SEQUENCE LISTING (67 sequences)

SEQ ID NO: 1 - DNA, 591 bp, Artificial Sequence
  DCW1
ttctaaaaccgtgactgcggatatcccgattgtgggggatgctcgccaggtcctcgaacaaatgcttgaactcttgtcgcaagaatccgcccatcaaccactggatgagatccgcgactggtggcagcaaattgaacagtggcgcgctcgtcagtgcctgaaatatgacactcacagtgaaaagattaaaccgcaggcggtgatcgagactctttggcggttgacgaagggagacgcttacgtgacgtccgatgtcgggcagcaccagatgtttgctgcactttattatccattcgacaaaccgcgtcgctggatcaattccggtggcctcggcacgatgggttttggtttacctgcggcactgggcgtcaaaatggcgttgccagaagaaaccgtggtttgcgtcactggcgacggcagtattcagatgaacatccaggaactgtctaccgcgttgcaatacgagttgcccgtactggtggtgaatctcaataaccgctatctggggatggtgaagcagtggcaggacatgatctattccggccgtcattcacaatcttatatgcaatcgctacccgatttcgtccgtct

SEQ ID NO: 2 - DNA, 591 bp, Artificial Sequence
  DCW2
gatctattccggccgtcattcacaatcttatatgcaatcgctacccgatttcgtccgtctggcggaagcctatgggcatgtcgggatccagatttctcatccgcatgagctggaaagcaaacttagcgaggcgctggaacaggtgcgcaataatcgcctggtgtttgttgatgttaccgtcgatggcagcgagcacgtctacccgatgcagattcgcgggggcggaatggatgaaatgtggttaagcaaaacggagagaacctgattatgcgccggatattatcagtcttactcgaaaatgaatcaggcgcgttatcccgcgtgattggccttttttcccagcgtggctacaacattgaaagcctgaccgttgcgccaaccgacgatccgacattatcgcgtatgaccatccagaccgtgggcgatgaaaaagtacttgagcagatcgaaaagcaattacacaaactggtcgatgtcttgcgcgtgagtgagttggggcagggcgcgcatgttgagcgggaaatcatgctggtgaaaattcaggccagcggttacgggcgtgacgaagtgaaacgtaatacggaaatattc

SEQ ID NO: 3 - DNA, 591 bp, Artificial Sequence
  DCW3
gtgaaaattcaggccagcggttacgggcgtgacgaagtgaaacgtaatacggaaatattccgtgggcaaattatcgatgtcacaccctcgctttataccgttcaattagcaggcaccagcggtaagcttgatgcatttttagcatcgattcgcgatgtggcgaaaattgtggaggttgctcgctctggtgtggtcggactttcgcgcggcgataaaataatgcgttgagaatgatctcaatgcgcaatttacagcccaacatgtcacgttgggctttttttgcgaaatcagtgggaacctggaataaaagcagttgccgcagttaattttctgcgcttagatgttaatgaatttaacccataccagtacaatggctatggtttttacattttacgcaaggggcaattgtgaaactggatgaaatcgctcggctggcgggagtgtcgcggaccactgcaagctatgttattaacggcaaagcgaagcaataccgtgtgagcgacaaaaccgttgaaaaagtcatggctgtggtgcgtgagcacaattaccacccgaacgccgtggcagctgggcttcgtgctggacgcacac

SEQ ID NO: 4 - DNA, 591 bp, Artificial Sequence
  DCW4
tgcgtgagcacaattaccacccgaacgccgtggcagctgggcttcgtgctggacgcacacgttctattggtcttgtgatccccgatctggagaacaccagctatacccgcatcgctaactatcttgaacgccaggcgcggcaacggggttatcaactgctgattgcctgctcagaagatcagccagacaacgaaatgcggtgcattgagcaccttttacagcgtcaggttgatgccattattgtttcgacgtcgttgcctcctgagcatcctttttatcaacgctgggctaacgacccgttcccgattgtcgcgctggaccgcgccctcgatcgtgaacacttcaccagcgtggttggtgccgatcaggatgatgccgaaatgctggcggaagagttacgtaagtttcccgccgagacggtgctttatcttggtgcgctaccggagctttctgtcagcttcctgcgtgaacaaggtttccgtactgcctggaaagatgatccgcgcgaagtgcatttcctgtatgccaacagctatgagcgggaggcggctgcccagttattcgaaaaatggctggaaacgcatccgatgc

SEQ ID NO: 5 - DNA, 591 bp, Artificial Sequence
  DCW5
gctatgagcgggaggcggctgcccagttattcgaaaaatggctggaaacgcatccgatgccgcaggcgctgttcacaacgtcgtttgcgttgttgcaaggagtgatggatgtcacgctgcgtcgcgacggcaaactgccttctgacctggcaattgccacctttggcgataacgaactgctcgacttcttacagtgtccggtgctggcagtggctcaacgtcaccgcgatgtcgcagagcgtgtgctggagattgtcctggcaagcctggacgaaccgcgtaagccaaaacctggtttaacgcgcattaaacgtaatctctatcgccgcggcgtgctcagccgtagctaagccgcgaacaaaaatacgcgccaggtgaatttccctctggcgcgtagagtacgggactggacatcaatatgcttaaagtaaataagactattcctgactattattgataaatgcttttaaacccgcccgttaattaactcaccagctgaaattcacaataattaagtgatatcgacagcgcgtttttgcattattttgttacatgcggcgatgaattgccgatttaacaaacacttttctt

SEQ ID NO: 6 - DNA, 591 bp, Artificial Sequence
  DCW6
gtttttgcattattttgttacatgcggcgatgaattgccgatttaacaaacacttttctttgcttttgcgcaaacccgctggcatcaagcgccacacagacgtaacaaggactgttaaccggggaagatatgtcctaaaatgccgctcgcgtcgcaaactgacactttatatttgctgtggaaaatagtgagtcattttaaaacggtgatgacgatgagggattttttcttacagctattcataacgttaatttgcttcgcacgttggacgtaaaataaacaacgctgatattagccgtaaacatcgggttttttacctcggtatgccttgtgactggcttgacaagcttttcctcagctccgtaaactcctttcagtgggaaattgtggggcaaagtgggaataaggggtgaggctggcatgttccggggagcaacgttagtcaatctcgacagcaaagggcgcttatcagtgcctacccgttatcgggaacagctgcttgagaacgctgccggtcaaatggtttgcaccattgacatttatcacccgtgcctgctgctttaccccctgcctgaatgggaaattatcgag

SEQ ID NO: 7 - DNA, 591 bp, Artificial Sequence
  DCW7
attgacatttatcacccgtgcctgctgctttaccccctgcctgaatgggaaattatcgagcaaaaattatcgcgtctgtcgagcatgaacccggttgagcgccgtgtgcagcgcctactgttaggtcatgccagcgaatgtcagatggatggcgcaggtcgattgttaatcgcgccagtactgcggcaacatgccgggctgacaaaagaagtgatgctggttggacagttcaacaagtttgagctgtgggatgaaacaacctggcatcaacaggtcaaggaagatatcgacgcagagcagttggctaccggagacttatcggagcgactgcaggacttgtctctataaaatgatggaaaactataaacatactacggtgctgctggatgaagccgttaatggcctcaatatccgtcctgatggcatctacattgatgggacttttggtcgcggtggtcactcacgtctgatcctctcgcagcttggcgaagaggggcgtttgctggcgatcgatcgcgacccgcaggctatcgccgttgcgaagactattgatgatccgcgcttctccatcatccacggacctttctccgc

SEQ ID NO: 8 - DNA, 591 bp, Artificial Sequence
  DCW8
cgccgttgcgaagactattgatgatccgcgcttctccatcatccacggacctttctccgcgctgggcgaatacgttgccgagcgcgatcttatcggcaagatcgacggcattctcctcgatcttggcgtctcttcaccgcaacttgatgatgctgaacgtggcttttcctttatgcgcgatggtccgctggacatgcgtatggacccaacccgtgggcagtcagccgctgaatggctacaaaccgcagaagaagccgatatcgcctgggtattgaaaacctatggtgaagagcgttttgccaaacgcattgcccgcgccattgtcgagcgtaaccgcgaacagccgatgacccgcaccaaagaactggcggaagtcgtggctgctgcaacgccggtgaaagataagtttaaacatcccgcgacccgtaccttccaggcggtgcgcatttgggtaaacagtgaactggaggagatagagcaggcgctaaaaagctcgctcaacgtgctggccccgggtgggcggctttcgatcatcagcttccactcgctggaagaccgtattgtgaaacgttttatgcgtgaaaacagccg

SEQ ID NO: 9 - DNA, 591 bp, Artificial Sequence
  DCW9
catcagcttccactcgctggaagaccgtattgtgaaacgttttatgcgtgaaaacagccgcggtccgcaagttccggcagggttaccgatgactgaagagcagctcaaaaaactgggtggccgtcagctgcgagcactaggcaagttaatgccgggcgaagaagaggtggctgagaaccctcgtgcccgtagttcagttctgcgtattgcagagaggacgaatgcatgatcagcagagtgacagaagctctaagcaaagttaaaggatcgatgggaagccacgagcgccatgcattgcctggtgttatcggtgacgatcttttgcgatttgggaagctgccactctgcctgttcatttgcattattttgacggcggtgactgtggtaaccacggcgcaccatacccgtttactgaccgctcagcgcgaacaactggtgctggagcgagatgctttagacattgaatggcgcaacctgatccttgaagagaatgcgctcggcgaccatagccgggtggaaaggatcgccacggaaaagctgcaaatgcagcatgttgatccgtcacaagaaaatatcgtagtgcaaaaataa

SEQ ID NO: 10 - DNA, 591 bp, Artificial Sequence
  DCW10
gaaaagctgcaaatgcagcatgttgatccgtcacaagaaaatatcgtagtgcaaaaataaggataaacgcgacgcatgaaagcagcggcgaaaacgcagaaaccaaaacgtcaggaagaacatgccaactttatcagttggcgttttgcgttgttatgcggctgtattctcctggcgctggcttttctgctcggacgcgtagcgtggttacaagttatctccccggatatgctggtgaaagagggcgacatgcgttctcttcgcgttcagcaagtttccacctcccgcggcatgattactgaccgttctggtcgcccgttagcggtgagcgtgccggtaaaagcgatttgggctgacccgaaagaagtgcatgacgctggcggtatcagcgtcggtgaccgctggaaggcgctggctaacgcgctcaatattccgctggatcagctttcagcccgcattaacgccaacccgaaagggcgctttatttatctggcgcgtcaggtgaaccctgacatggcggactacatcaaaaaactgaaactgccggggattcatctgcgtgaagagtctcgccgttactatccgtccggc

SEQ ID NO: 11 - DNA, 591 bp, Artificial Sequence
  DCW11
aaactgaaactgccggggattcatctgcgtgaagagtctcgccgttactatccgtccggcgaagtgactgctcacctcatcggctttactaacgtcgatagtcaagggattgagggcgttgagaagagtttcgataaatggcttaccgggcagccgggtgagcgcattgtgcgtaaagaccgctatggtcgcgtaattgaagatatttcttctactgacagccaggcagcgcacaacctggcgctgagtattgatgaacgcctgcaggcgctggtttatcgcgaactgaacaacgcggtggcctttaacaaggctgaatctggtagcgccgtgctggtggatgtcaacaccggtgaagtgctggcgatggctaacagcccgtcatacaaccctaacaatctgagcggcacgccgaaagaggcgatgcgtaaccgtaccatcaccgacgtgtttgaaccgggctcaacggttaaaccgatggtggtaatgaccgcgttgcaacgtggcgtggtgcgggaaaactcggtactcaataccattccttatcgaattaacggccacgaaatcaaagacgtggcacgctacagcgaa

SEQ ID NO: 12 - DNA, 591 bp, Artificial Sequence
  DCW12
aataccattccttatcgaattaacggccacgaaatcaaagacgtggcacgctacagcgaattaaccctgaccggggtattacagaagtcgagtaacgtcggtgtttccaagctggcgttagcgatgccgtcctcagcgttagtagatacttactcacgttttggactgggaaaagcgaccaatttggggttggtcggagaacgcagtggcttatatcctcaaaaacaacggtggtctgacatagagagggccaccttctctttcggctacgggctaatggtaacaccattacagttagcgcgagtctacgcaactatcggcagctacggcatttatcgcccactgtcgattaccaaagttgaccccccggttcccggtgaacgtgtcttcccggaatccattgtccgcactgtggtgcatatgatggaaagcgtggcgctaccaggcggcggcggcgtgaaggcggcgattaaaggctatcgtatcgccattaaaaccggtaccgcgaaaaaggtcgggccggacggtcgctacatcaataaatatattgcttataccgcaggcgttgcgcctgcgagtcagccgcgcttc

SEQ ID NO: 13 - DNA, 571 bp, Artificial Sequence
  DCW13b
taaatatattgcttataccgcaggcgttgcgcctgcgagtcagccgcgcttcgcgctggttgttgttatcaacgatccgcaggcgggtaaatactacggcggcgccgtttccgcgccggtctttggtgccatcatgggcggcgtattgcgtaccatgaacatcgagccggatgcgctgacaacgggcgataaaaatgaatttgtgattaatcaaggcgaggggacaggtggcagatcgtaatttgcgcgaccttcttgctccgtgggtgccagacgcaccttcgcgagcactgcgagagatgacactcgacagccgtgtggctgcggcgggcgatctctttgtagctgtagtaggtcatcaggcggacgggcgtcgatatatcccgcaggcgatagcgcaaggtgtggctgccattattgcagaggcgaaagatgaggcgaccgatggtgaaatccgtgaaatgcacggcgtaccggtcatctatctcagccagctcaacgagcgtttatctgcactggcgggccgcttttaccatgaaccctctgacaatttacgtctcgtgggcgtaac

SEQ ID NO: 14 - DNA, 591 bp, Artificial Sequence
  DCW14
ccgcttttaccatgaaccctctgacaatttacgtctcgtgggcgtaacgggcaccaacggcaaaaccacgactacccagctgttggcgcagtggagccaactgcttggcgaaatcagcgcggtaatgggcaccgttggtaacggcctgctggggaaagtgatcccgacagaaaatacaaccggttcggcagtcgatgttcagcatgagctggcggggctggtggatcagggcgcgacgttttgcgcaatggaagtttcctcccacgggctggtacagcaccgtgtggcggcattgaaatttgcggcgtcggtctttaccaacttaagccgcgatcaccttgattatcatggtgatatggaacactacgaagccgcgaaatggctgctttattctgagcatcattgcggtcaggcgattattaacgccgacgatgaagtgggccgccgctggctggcaaaactgccggacgcggttgcggtatcaatggaagatcatattaatccgaactgtcacggacgctggttgaaagcgaccgaagtgaactatcacgacagcggtgcgacgattcgctttagctcaagttggggcga

SEQ ID NO: 15 - DNA, 591 bp, Artificial Sequence
  DCW15
gaccgaagtgaactatcacgacagcggtgcgacgattcgctttagctcaagttggggcgatggcgaaattgaaagccatctgatgggcgcttttaacgtcagcaacctgctgctcgcgctggcgacactgttggcactcggctatccactggctgatctgctgaaaaccgccgcgcgtctgcaaccggtttgcggacgtatggaagtgttcactgcgccaggcaaaccgacggtggtggtggattacgcgcatacgccggatgcactggaaaaagccttacaggcggcgcgtctgcactgtgcgggcaagctgtggtgtgtctttggctgtggtggcgatcgcgataaaggtaagcgtccactgatgggcgcaattgccgaagagtttgctgacgtggcggtggtgacggacgataacccgcgtaccgaagaaccgcgtgccatcatcaacgatattctggcgggaatgttagatgccggacatgccaaagtgatggaaggccgtgctgaagcggtgacttgcgccgttatgcaggctaaagagaatgatgtggtactggtcgcgggcaaaggccatgaagattaccagat

SEQ ID NO: 16 - DNA, 591 bp, Artificial Sequence
  DCW16
gcaggctaaagagaatgatgtggtactggtcgcgggcaaaggccatgaagattaccagattgttggcaatcagcgtctggactactccgatcgcgtcacggtggcgcgtctgctgggggtgattgcatgattagcgtaacccttagccaacttaccgacattctcaacggtgaactgcaaggtgcagatatcacccttgatgctgtaaccactgatacccgaaaactgacgccgggctgcctgtttgttgccctgaaaggcgaacgttttgatgcccacgattttgccgaccaggcgaaagctggcggcgcaggcgcactactggttagccgtccgctggacatcgacctgccgcagttaatcgtcaaggatacgcgtctggcgtttggtgaactggctgcatgggttcgccagcaagttccggcgcgcgtggttgctctgacggggtcctccggcaaaacctccgttaaagagatgacggcggcgattttaagccagtgcggcaacacgctttatacggcaggcaatctcaacaacgacatcggtgtaccgatgacgctgttgcgcttaacgccggaatacgattacgca

SEQ ID NO: 17 - DNA, 591 bp, Artificial Sequence
  DCW17
aacaacgacatcggtgtaccgatgacgctgttgcgcttaacgccggaatacgattacgcagttattgaacttggcgcgaaccatcagggcgaaatagcctggactgtgagtctgactcgcccggaagctgcgctggtcaacaacctggcagcggcgcatctggaaggttttggctcgcttgcgggtgtcgcgaaagcgaaaggtgaaatctttagcggcctgccggaaaacggtatcgccattatgaacgccgacaacaacgactggctgaactggcagagcgtaattggctcacgcaaagtgtggcgtttctcacccaatgccgccaacagcgatttcaccgccaccaatatccatgtgacctcgcacggtacggaatttaccctacaaaccccaaccggtagcgtcgatgttctgctgccgttgccggggcgtcacaatattgcgaatgcgctggcagccgctgcgctctccatgtccgtgggcgcaacgcttgatgctatcaaagcggggctggcaaatctgaaagctgttccaggccgtctgttccccatccaactggcagaaaaccagttgctgctcgacgactcc

SEQ ID NO: 18 - DNA, 591 bp, Artificial Sequence
  DCW18
gttccaggccgtctgttccccatccaactggcagaaaaccagttgctgctcgacgactcctacaacgccaatgtcggttcaatgactgcagcagtccaggtactggctgaaatgccgggctaccgcgtgctggtggtgggcgatatggcggaactgggcgctgaaagcgaagcctgccatgtacaggtgggcgaggcggcaaaagctgctggtattgaccgcgtgttaagcgtgggtaaacaaagccatgctatcagcaccgccagcggcgttggcgaacattttgctgataaaactgcgttaattacgcgtcttaaattactgattgctgagcaacaggtaattacgattttagttaagggttcacgtagtgccgccatggaagaggtagtacgcgctttacaggagaatgggacatgttagtttggctggccgaacatttggtcaaatattattccggctttaacgtcttttcctatctgacgtttcgcgccatcgtcagcctgctgaccgcgctgttcatctcattgtggatgggcccgcgtatgattgctcatttgcaaaaactttcctttggtcaggtggtgcgta

SEQ ID NO: 19 - DNA, 591 bp, Artificial Sequence
  DCW19
ggatgggcccgcgtatgattgctcatttgcaaaaactttcctttggtcaggtggtgcgtaacgacggtcctgaatcacacttcagcaagcgcggtacgccgaccatgggcgggattatgatcctgacggcgattgtgatctccgtactgctgtgggcttacccgtccaatccgtacgtctggtgcgtgttggtggtgctggtaggttacggtgttattggctttgttgatgattatcgcaaagtggtgcgtaaagacaccaaagggttgatcgctcgttggaagtatttctggatgtcggtcattgcgctgggtgtcgccttcgccctgtaccttgccggcaaagacacgcccgcaacgcagctggtggtcccattctttaaagatgtgatgccgcagctggggctgttctacattctgctggcttacttcgtcattgtgggtactggcaacgcggtaaacctgaccgatggtctcgacggcctggcaattatgccgaccgtatttgtcgccggtggttttgcgctggtggcgtgggcgaccggcaatatgaactttgccagctacttgcatataccgtatctgcgacacg

SEQ ID NO: 20 - DNA, 591 bp, Artificial Sequence
  DCW20
cgtgggcgaccggcaatatgaactttgccagctacttgcatataccgtatctgcgacacgccggggaactggttattgtctgtaccgcgatagtcggggcaggactgggcttcctgtggtttaacacctatccggcgcaggtctttatgggcgatgtaggttcgctggcgttaggtggtgcgttaggcattatcgccgtactgctacgtcaggaattcctgctggtgattatggggggcgtgttcgtggtagaaacgctttctgtcatcctgcaggtcggctcctttaaactgcgcggacaacgtattttccgcatggcaccgattcatcaccactatgaactgaaaggctggccggaaccgcgcgtcattgtgcgtttctggattatttcgctgatgctggttctgattggtctggcaacgctgaaggtacgttaatcatggctgattatcagggtaaaaatgtcgtcattatcggcctgggcctcaccgggctttcctgcgtggactttttcctcgctcgcggtgtgacgccgcgcgttatggatacgcgtatgacaccgcctggcctggataaattacccgaagccgt

SEQ ID NO: 21 - DNA, 591 bp, Artificial Sequence
  DCW21
gccgcgcgttatggatacgcgtatgacaccgcctggcctggataaattacccgaagccgtagaacgccacacgggcagtctgaatgatgaatggctgatggcggcagatctgattgtcgccagtcccggtattgcactggcgcatccatccttaagcgctgccgctgatgccggaatcgaaatcgttggcgatatcgagctgttctgtcgcgaagcacaagcaccgattgtggcgattaccggttctaacggcaaaagcacggtcaccacgctagtgggtgaaatggcgaaagcggcgggggttaacgttggtgtgggtggcaatattggcctgcctgcgttgatgctactggatgatgagtgtgaactgtacgtgctggaactgtcgagcttccagctggaaaccacctccagcttacaggcggtagcagcgaccattctgaacgtgactgaagatcatatggatcgctatccgtttggtttacaacagtatcgtgcagcaaaactgcgcatttacgaaaacgcgaaagtttgcgtggttaatgctgatgatgccttaacaatgccgattcgcggtgcggatgaacgctg

SEQ ID NO: 22 - DNA, 591 bp, Artificial Sequence
  DCW22
ttgcgtggttaatgctgatgatgccttaacaatgccgattcgcggtgcggatgaacgctgcgtcagctttggcgtcaacatgggtgactatcacctgaatcatcagcagggcgaaacctggctgcgggttaaaggcgagaaagtgctgaatgtgaaagagatgaaactttccgggcagcataactacaccaatgcgctggcggcgctggcgctggcagatgctgcagggttaccgcgtgccagcagcctgaaagcgttaaccacattcactggtctgccgcatcgctttgaagttgtgctggagcataacggcgtacgttggattaacgattcgaaagcgaccaacgtcggcagtacggaagcggcgctgaatggcctgcacgtagacggcacactgcatttgttgctgggtggcgatggtaaatcggcggactttagcccactggcgcgttacctgaatggcgataacgtacgtctgtattgtttcggtcgtgacggcgcgcagctggcggcgctacgcccggaagtggcagaacaaaccgaaactatggaacaggcgatgcgcttgctggctccgcgtgttcagccggg

SEQ ID NO: 23 - DNA, 591 bp, Artificial Sequence
  DCW23
agaacaaaccgaaactatggaacaggcgatgcgcttgctggctccgcgtgttcagccgggcgatatggttctgctctccccagcctgtgccagccttgatcagttcaagaactttgaacaacgaggcaatgagtttgcccgtctggcgaaggagttaggttgatgcgtttatctctccctcgcctgaaaatgccgcgcctgccaggattcagtatcctggtctggatctccacggcgctaaagggctgggtgatgggctcgcgggaaaaagataccgacagcctgatcatgtacgatcgcaccttactgtggctgaccttcggcctcgcggcgattggctttatcatggtgacctcggcgtcaatgcccatagggcaacgcttaaccaacgatccgttcttcttcgcgaagcgtgatggtgtctatctgattttggcgtttattctggcgatcattacgctgcgtctgccgatggagttctggcaacgctacagtgccacgatgctgctcggatctatcatcctgctgatgatcgtcctggtagtgggtagctcggttaaaggggcatcgcgttggatcgatctcggtttg

SEQ ID NO: 24 - DNA, 589 bp, Artificial Sequence
  DCW24b
atcgtcctggtagtgggtagctcggttaaaggggcatcgcgttggatcgatctcggtttgctgcgtatccagcctgcggagctgacaaaactgtcgctgttttgctatatcgccaactatctggtgcgtaaaggcgacgaagtacgtaataacctgcgcggcttcctgaaaccgatgggcgtgattctggtgttggcagtgttactgctggcacagccagaccttggtacggtggtggtgttgtttgtgactacgctggcgatgttgttcctggcgggagcgaaattgtggcagttcattgccattatcggtatgggcatttcagcggttgtgttgctgatactcgccgaaccgtaccgtatccgccgtgttaccgcattctggaacccgtgggaagatccctttggcagcggctatcagttaacgcaatcgctgatggcgtttggtcgcggcgaactttgggggcaaggtttaggtaactcggtacaaaaactggagtatctgccggaagcgcacactgactttattttcgccattatcggcgaagaactggggtatgtcggtgtggtgctggcacttttaatggtat

SEQ ID NO: 25 - DNA, 591 bp, Artificial Sequence
  DCW25
gccattatcggcgaagaactggggtatgtcggtgtggtgctggcacttttaatggtattcttcgtcgcttttcgcgcgatgtcgattggccgtaaagcattagaaattgaccaccgtttttccggttttctcgcctgttctattggcatctggtttagcttccaggcgctggttaacgtaggcgcggcggcggggatgttaccgaccaaaggtctgacattgccgctgatcagttacggtggttcgagcttactgattatgtcgacagccatcatgatgctgttgcgtattgattatgaaacgcgtctggagaaagcgcaggcgtttgtacgaggttcacgatgagtggtcaaggaaagcgattaatggtgatggcaggcggaaccggtggacatgtattcccgggactggcggttgcgcaccatctaatggctcagggttggcaagttcgctggctggggactgccgaccgtatggaagcggacttagtgccaaaacatggcatcgaaattgatttcattcgtatctctggtctgcgtggaaaaggtataaaagcactgatagctgccccgctgcgtatcttcaacgcct

SEQ ID NO: 26 - DNA, 591 bp, Artificial Sequence
  DCW26
gtctgcgtggaaaaggtataaaagcactgatagctgccccgctgcgtatcttcaacgcctggcgtcaggcgcgggcgattatgaaagcgtacaaacctgacgtggtgctcggtatgggaggctacgtgtcaggtccaggtggtctggccgcgtggtcgttaggcattccggttgtacttcatgaacaaaacggtattgcgggcttaaccaataaatggctggcgaagattgccaccaaagtgatgcaggcgtttccaggtgctttccctaatgcggaagtagtgggtaacccggtgcgtaccgatgtgttggcgctgccgttgccgcagcaacgtttggctggacgtgaaggtccggttcgtgtgctggtagtgggtggttctcagggcgcacgcattcttaaccagacaatgccgcaggttgctgcgaaactgggtgattcagtcactatctggcatcagagcggcaaaggttcgcaacaatccgttgaacaggcgtatgccgaagcggggcaaccgcagcataaagtgacggaatttattgatgatatggcggcggcgtatgcgtgggcggatgtcgtcgtttgccgct

SEQ ID NO: 27 - DNA, 591 bp, Artificial Sequence
  DCW27
cggaatttattgatgatatggcggcggcgtatgcgtgggcggatgtcgtcgtttgccgctccggtgcgttaacggtgagtgaaatcgccgcggcaggactaccggcgttgtttgtgccgtttcaacataaagaccgccagcaatactggaatgcgctaccgctggaaaaagcgggcgcagccaaaattatcgagcagccacagcttagcgtggatgctgtcgccaacaccctggccgggtggtcgcgagaaaccttattaaccatggcagaacgcgcccgcgctgcatccattccggatgccaccgagcgagtggcaaatgaagtgagccgggttgcccgggcgtaattgtagcgatgccttttgcatcgtatgaatttaagaagttaatggcgtaaagaatgaatacacaacaattggcaaaactgcgttccatcgtgcccgaaatgcgtcgcgttcggcacatacattttgtcggcattggtggtgccggtatgggcggtattgccgaagttctggccaatgaaggttatcagatcagtggttccgatttagcgccaaatccggtcacgcagcagttaatgaatctggg

SEQ ID NO: 28 - DNA, 591 bp, Artificial Sequence
  DCW28
tcagatcagtggttccgatttagcgccaaatccggtcacgcagcagttaatgaatctgggtgcgacgatttatttcaaccatcgcccggaaaacgtacgtgatgccagcgtggtcgttgtttccagcgcgatttctgccgataacccggaaattgtcgccgctcatgaagcgcgtattccggtgatccgtcgtgccgaaatgctggctgagttaatgcgttttcgtcatggcatcgccattgccggaacgcacggcaaaacgacaaccaccgcgatggtttccagcatctacgcagaagcggggctcgacccaaccttcgttaacggcgggctggtaaaagcggcgggggttcatgcgcgtttggggcatggtcggtacctgattgccgaagcagatgagagtgatgcatcgttcctgcatctgcaaccgatggtggcgattgtcaccaatatcgaagccgaccacatggatacctaccagggcgactttgagaatttaaaacagacttttattaattttctgcacaacctgccgttttacggtcgtgcggtgatgtgtgttgatgatccggtgatccgcgaattgttacc

SEQ ID NO: 29 - DNA, 591 bp, Artificial Sequence
  DCW29
gccgttttacggtcgtgcggtgatgtgtgttgatgatccggtgatccgcgaattgttaccgcgagtggggcgtcagaccacgacttacggcttcagcgaagatgccgacgtgcgtgtagaagattatcagcagattggcccgcaggggcactttacgctgctgcgccaggacaaagagccgatgcgcgtcaccctgaatgcgccaggtcgtcataacgcgctgaacgccgcagctgcggttgcggttgctacggaagagggcattgacgacgaggctattttgcgggcgcttgaaagcttccaggggactggtcgccgttttgatttcctcggtgaattcccgctggagccagtgaatggtaaaagcggtacggcaatgctggtcgatgactacggccaccacccgacggaagtggacgccaccattaaagcggcgcgcgcaggctggccggataaaaacctggtaatgctgtttcagccgcaccgttttacccgtacgcgcgacctgtatgatgatttcgccaatgtgctgacgcaggttgataccctgttgatgctggaagtgtatccggctggcgaagcgccaattcc

SEQ ID NO: 30 - DNA, 591 bp, Artificial Sequence
  DCW30
gacgcaggttgataccctgttgatgctggaagtgtatccggctggcgaagcgccaattccgggagcggacagccgttcgctgtgtcgcacaattcgtggacgtgggaaaattgatcccattctggtgccggatccggcgcgggtagccgagatgctggcaccggtattaaccggtaacgacctgattctcgttcagggggctggtaatattggaaaaattgcccgttctttagctgaaatcaaactgaagccgcaaactccggaggaagaacaacatgactgataaaatcgcggtcctgttgggtgggacctccgctgagcgggaagtttctctgaattctggcgcagcggtgttagccggactgcgtgaaggcggtattgacgcgtatcctgtcgacccgaaagaagtcgacgtgacgcaactgaagtcgatgggctttcagaaagtgtttatcgcgctacacggtcgcggcggtgaagatggtacgctgcaggggatgctcgagctgatgggcttgccttataccggaagcggagtgatggcatctgcgctttcaatggataaactacgcagcaaacttctatggcaag

SEQ ID NO: 31 - DNA, 591 bp, Artificial Sequence
  DCW31
gcggagtgatggcatctgcgctttcaatggataaactacgcagcaaacttctatggcaaggtgccggtttaccggtcgcgccgtgggtagcgttaacccgcgcagagtttgaaaaaggcctgagcgataagcagttagcagaaatttctgctctgggtttgccggttatcgttaagccgagccgcgaaggttccagtgtgggaatgtcaaaagtagtagcagaaaatgctctacaagatgcattaagattggcatttcagcacgatgaagaagtattgattgaaaaatggctaagtgggccggagttcacggttgcgatactcggtgaagaaattttaccgtcaatacgtattcaaccgtccggaaccttctatgattatgaggcgaagtatctctctgatgagacacagtatttctgccccgcaggtctggaagcgtcacaagaggccaatttgcaggcattagtgctgaaagcatggacgacgttaggttgcaaaggatggggacgtattgacgttatgctggacagcgatggacagttttatctgctggaagccaatacctcaccgggtatgaccagccacagcctgg

SEQ ID NO: 32 - DNA, 579 bp, Artificial Sequence
  DCW32b
atggacagttttatctgctggaagccaatacctcaccgggtatgaccagccacagcctggtgccgatggcggcacgtcaggcaggtatgagcttctcgcagttggtagtacgaattctggaactggcggactaatatgtcgcaggctgctctgaacacgcgaaacagcgaagaagaggtttcttctcgccgcaataatggaacgcgtctggcggggatccttttcctgctgaccgttttaacgacagtgttggtgagcggctgggtcgtgttgggctggatggaagatgcgcaacgcctgccgctctcaaagctggtgttgaccggtgaacgccattacacacgtaatgacgatatccggcagtcgatcctggcattgggtgagccgggtacctttatgacccaggatgtcaacatcatccagacgcaaatagaacaacgcctgccgtggattaagcaggtgagcgtcagaaagcagtggcctgatgaattgaagattcatctggttgaatatgtgccgattgcgcggtggaatgatcaacatatggtagacgcggaaggaaataccttcagcgtgccg

SEQ ID NO: 33 - DNA, 591 bp, Artificial Sequence
  DCW33
aatgatcaacatatggtagacgcggaaggaaataccttcagcgtgccgccagaacgcaccagcaagcaggtgcttccaatgctgtatggcccggaaggcagcgccaatgaagtgttgcagggctatcgcgaaatggggcagatgctggcaaaggacagatttactctgaaggaagcggcgatgaccgcgcggcgttcctggcagttgacgctgaataacgatattaagctcaatcttggccggggcgatacgatgaaacgtttggctcgctttgtagaactttatccggttttacagcagcaggcgcaaaccgatggcaaacggattagctacgttgatttgcgttatgactctggagcggcagtaggctgggcgcccttgccgccagaggaatctactcagcaacaaaatcaggcacaggcagaacaacaatgatcaaggcgacggacagaaaactggtagtaggactggagattggtaccgcgaaggttgccgctttagtaggggaagttctgcccgacggtatggtcaatatcattggcgtgggcagctgcccgtcgcgtggtatggataaaggcggggtgaacgacc

SEQ ID NO: 34 - DNA, 591 bp, Artificial Sequence
  DCW34
atatcattggcgtgggcagctgcccgtcgcgtggtatggataaaggcggggtgaacgacctcgaatccgtggtcaagtgcgtacaacgcgccattgaccaggcagaattgatggcagattgtcagatctcttcggtatatctggcgctttctggtaagcacatcagctgccagaatgaaattggtatggtgcctatttctgaagaagaagtgacgcaagaagatgtggaaaacgtcgtccataccgcgaaatcggtgcgtgtgcgcgatgagcatcgtgtgctgcatgtgatcccgcaagagtatgcgattgactatcaggaagggatcaagaatccggtaggactttcgggcgtgcggatgcaggcaaaagtgcacctgatcacatgtcacaacgatatggcgaaaaacatcgtcaaagcggttgaacgttgtgggctgaaagttgaccaactgatatttgccggactggcatcaagttattcggtattgacggaagatgaacgtgaactgggtgtctgcgtcgtcgatatcggtggtggtacaatggatatcgccgtttataccggtggggcattgcgccacactaagg

SEQ ID NO: 35 - DNA, 591 bp, Artificial Sequence
  DCW35
tcggtggtggtacaatggatatcgccgtttataccggtggggcattgcgccacactaaggtaattccttatgctggcaatgtcgtgaccagtgatatcgcttacgcctttggcacgccgccaagcgacgccgaagcgattaaagttcgccacggttgtgcgctgggttccatcgttggaaaagatgagagcgtggaagtgccgagcgtaggtggtcgtccgccacggagtctgcaacgtcagacactggcagaggtgatcgagccgcgctataccgagctgctcaacctggtcaacgaagagatattgcagttgcaggaaaagcttcgccaacaaggggttaaacatcacctggcggcaggcattgtattaaccggtggcgcagcgcagatcgaaggtcttgcagcctgtgctcagcgcgtgtttcatacgcaagtgcgtatcggcgcgccgctgaacattaccggtttaacggattatgctcaggagccgtattattcgacggcggtgggattgcttcactatgggaaagagtcacatcttaacggtgaagctgaagtagaaaaacgtgttacagcatcagttggctcgt

SEQ ID NO: 36 - DNA, 591 bp, Artificial Sequence
  DCW36
agtcacatcttaacggtgaagctgaagtagaaaaacgtgttacagcatcagttggctcgtggatcaagcgactcaatagttggctgcgaaaagagttttaatttttatgaggccgacgatgattacggcctcaggcgacaggcacaaatcggagagaaactatgtttgaaccaatggaacttaccaatgacgcggtgattaaagtcatcggcgtcggcggcggcggcggtaatgctgttgaacacatggtgcgcgagcgcattgaaggtgttgaattcttcgcggtaaataccgatgcacaagcgctgcgtaaaacagcggttggacagacgattcaaatcggtagcggtatcaccaaaggactgggcgctggcgctaatccagaagttggccgcaatgcggctgatgaggatcgcgatgcattgcgtgcggcgctggaaggtgcagacatggtctttattgctgcgggtatgggtggtggtaccggtacaggtgcagcaccagtcgtcgctgaagtggcaaaagatttgggtatcctgaccgttgctgtcgtcactaagcctttcaactttgaaggcaagaagcgtatgg

SEQ ID NO: 37 - DNA, 591 bp, Artificial Sequence
  DCW37
gtatcctgaccgttgctgtcgtcactaagcctttcaactttgaaggcaagaagcgtatggcattcgcggagcaggggatcactgaactgtccaagcatgtggactctctgatcactatcccgaacgacaaactgctgaaagttctgggccgcggtatctccctgctggatgcgtttggcgcagcgaacgatgtactgaaaggcgctgtgcaaggtatcgctgaactgattactcgtccgggtttgatgaacgtggactttgcagacgtacgcaccgtaatgtctgagatgggctacgcaatgatgggttctggcgtggcgagcggtgaagaccgtgcggaagaagctgctgaaatggctatctcttctccgctgctggaagatatcgacctgtctggcgcgcgcggcgtgctggttaacatcacggcgggcttcgacctgcgtctggatgagttcgaaacggtaggtaacaccatccgtgcatttgcttccgacaacgcgactgtggttatcggtacttctcttgacccggatatgaatgacgagctgcgcgtaaccgttgttgcgacaggtatcggcatggacaaacgtc

SEQ ID NO: 38 - DNA, 591 bp, Artificial Sequence
  DCW38
atatgaatgacgagctgcgcgtaaccgttgttgcgacaggtatcggcatggacaaacgtcctgaaatcactctggtgaccaataagcaggttcagcagccagtgatggatcgctaccagcagcatgggatggctccgctgacccaggagcagaagccggttgctaaagtcgtgaatgacaatgcgccgcaaactgcgaaagagccggattatctggatatcccagcattcctgcgtaagcaagctgattaagaattgactggaatttgggtttcgaggctctttgtgctaaactggcccgccgaatgtatagtacacttcggttggataggtaatttggcgagataatacgatgatcaaacaaaggacacttaaacgtatcgttcaggcgacgggtgtcggtttacataccggcaagaaagtcaccctgacgttacgccctgcgccggccaacaccggggtcatctatcgtcgcaccgacttgaatccaccggtagatttcccggccgatgccaaatctgtgcgtgataccatgctctgtacgtgtctggtcaacgagcatgatgtacggatttcaaccgtagagcacctc

SEQ ID NO: 39 - DNA, 591 bp, Artificial Sequence
  DCW39
atgctctgtacgtgtctggtcaacgagcatgatgtacggatttcaaccgtagagcacctcaatgctgctctcgcgggcttgggcatcgataacattgttatcgaagttaacgcgccggaaatcccgatcatggacggcagcgccgctccgtttgtatacctgctgcttgacgccggtatcgacgagttgaactgcgccaaaaaatttgttcgcatcaaagagactgttcgtgtcgaagatggcgataagtgggctgaatttaagccgtacaatggtttttcgctggatttcaccatcgattttaaccatccggctattgattccagcaaccagcgctatgcgatgaacttctccgctgatgcgtttatgcgccagatcagccgtgcgcgtacgttcggtttcatgcgtgatatcgaatatctgcagtcccgtggtttgtgcctgggcggcagcttcgattgtgccatcgttgttgacgattatcgcgtactgaacgaagacggcctgcgttttgaagacgaatttgtgcgtcacaaaatgctcgatgcgatcggtgacttgttcatgtgtggtcacaatattattggtgca

SEQ ID NO: 40 - DNA, 591 bp, Artificial Sequence
  DCW40
cacaaaatgctcgatgcgatcggtgacttgttcatgtgtggtcacaatattattggtgcatttaccgcttataaatccggtcatgcactgaataacaaactgctgcaggctgtcctggcgaaacaggaagcctgggaatatgtgaccttccaggacgacgcagaactgccgttggccttcaaagcgccttcagctgtactggcataacgacatttatactgtcgtataaaattcgactggcaaatctggcactctctccggccaggtgaaccagtcgtttttttttgaattttataagagctataaaaaacggtgcgaacgctgttttcttaagcacttttccgcacaacttatcttcattcgtgctgtggactgcaggctttaatgataagatttgtgcgctaaatacgtttgaatatgatcgggatggcaataacgtgagtggaatactgacgcgctggcgacagtttggtaaacgctacttctggccgcatctcttattagggatggttgcggcgagtttaggtttgcctgcgctcagcaacgccgccgaaccaaacgcgcccgcaaaagcgacaacccgcaaccacg

SEQ ID NO: 41 - DNA, 591 bp, Artificial Sequence
  DCW41
ctgcgctcagcaacgccgccgaaccaaacgcgcccgcaaaagcgacaacccgcaaccacgagccttcagccaaagttaactttggtcaattggccttgctggaagcgaacacacgccgcccgaattcgaactattccgttgattactggcatcaacatgccattcgcacggtaatccgtcatctttctttcgcaatggcaccgcaaacactgcccgttgctgaagaatctttgcctcttcaggcgcaacatcttgcattactggatacgctcagcgcgctgctgacccaggaaggcacgccgtctgaaaagggttatcgcattgattatgcgcattttaccccacaagcaaaattcagcacgcccgtctggataagccaggcgcaaggcatccgtgctggccctcaacgcctcacctaacaacaataaacctttacttcattttattaactccgcaacgcggggcgtttgagattttattatgctaatcaaattgttaactaaagttttcggtagtcgtaacgatcgcaccctgcgccggatgcgcaaagtggtcaacatcatcaatgccatggaaccggagatggaaaaa

SEQ ID NO: 42 - DNA, 591 bp, Artificial Sequence
  DCW42
ctgcgccggatgcgcaaagtggtcaacatcatcaatgccatggaaccggagatggaaaaactctccgacgaagaactgaaagggaaaaccgcagagtttcgtgcacgtctggaaaaaggcgaagtgctggaaaatctgatcccggaagctttcgccgtggtacgtgaggcaagtaagcgcgtctttggtatgcgtcacttcgacgttcagttactcggcggtatggttcttaacgaacgctgcatcgccgaaatgcgtaccggtgaaggaaaaaccctgaccgcaacgctgcctgcttacctgaacgcactaaccggtaaaggcgtgcacgtagttaccgtcaacgactacctggcgcaacgtgacgccgaaaacaaccgtccgctgtttgaattccttggcctgactgtcggtatcaacctgccgggcatgccagcaccggcaaagcgcgaagcttacgcagctgacatcacttacggtacgaacaacgaatacggctttgactacctgcgcgacaacatggcgttcagccctgaagaacgtgtacagcgtaaactgcactatgcgctggtggacgaagtggactccatc

SEQ ID NO: 43 - DNA, 591 bp, Artificial Sequence
  DCW43
cctgaagaacgtgtacagcgtaaactgcactatgcgctggtggacgaagtggactccatcctgatcgatgaagcgcgtacaccgctgatcatttccggcccggcagaagacagctcggaaatgtataaacgcgtgaataaaattattccgcacctgatccgtcaggaaaaagaagactccgaaaccttccagggcgaaggccacttctcggtggacgaaaaatctcgccaggtgaacctgaccgaacgtggtctggtgctgattgaagaactgctggtgaaagagggcatcatggatgaaggggagtctctgtactctccggccaacatcatgctgatgcaccacgtaacggcggcgctgcgcgctcatgcgctgtttacccgtgacgtcgactacatcgttaaagatggtgaagttatcatcgttgacgaacacaccggtcgtaccatgcagggccgtcgctggtccgatggtctgcaccaggctgtggaagcgaaagaaggtgtgcagatccagaacgaaaaccaaacgctggcttcgatcaccttccagaactacttccgtctgtatgaaaaactggcggggatgacc

SEQ ID NO: 44 - DNA, 591 bp, Artificial Sequence
  DCW44
ctggcttcgatcaccttccagaactacttccgtctgtatgaaaaactggcggggatgaccggtactgctgataccgaagctttcgaatttagctcaatctacaagctggataccgtcgttgttccgaccaaccgtccaatgattcgtaaagatctgccggacctggtctacatgactgaagcggaaaaaattcaggcgatcattgaagatatcaaagaacgtactgcgaaaggccagccggtgctggtgggtactatctccatcgaaaaatcggagctggtgtcaaacgaactgaccaaagccggtattaagcacaacgtcctgaacgccaaattccacgccaacgaagcggcgattgttgctcaggcaggttatccggctgcggtgactatcgcgaccaatatggcgggtcgtggtacagatattgtgctcggtggtagctggcaggcagaagttgccgcgctggaaaatccgaccgcagagcaaattgaaaaaattaaagccgactggcaggtacgtcacgatgcggtactggaagcaggtggcctgcatatcatcggtaccgagcgtcacgaatcccgtcgtatcgat

SEQ ID NO: 45 - DNA, 591 bp, Artificial Sequence
  DCW45
ctggaagcaggtggcctgcatatcatcggtaccgagcgtcacgaatcccgtcgtatcgataaccagttgcgcggtcgttctggtcgtcagggggatgctggttcttcccgtttctacctgtcgatggaagatgcgctgatgcgtatttttgcttccgaccgagtatccggcatgatgcgtaaactgggtatgaagccaggcgaagccattgaacacccgtgggtgactaaagcgattgccaacgcccagcgtaaagttgaaagccgtaacttcgacattcgtaagcaactgctggaatatgatgacgtggctaacgatcagcgtcgcgccatttactcccagcgtaacgaactgttggatgtcagcgatgtgagcgaaaccattaacagcattcgtgaagatgtgttcaaagcgaccattgatgcctacattccaccacagtcgctggaagaaatgtgggatattccggggctgcaggaacgtctgaagaacgatttcgacctcgatttgccaattgccgagtggctggataaagaaccagaactgcatgaagagacgctgcgtgagcgcattctggcgcagtccatcgaa

SEQ ID NO: 46 - DNA, 591 bp, Artificial Sequence
  DCW46
aaagaaccagaactgcatgaagagacgctgcgtgagcgcattctggcgcagtccatcgaagtgtatcagcgtaaagaagaagtggttggtgctgagatgatgcgtcacttcgagaaaggcgtcatgctgcaaacgcttgactccctgtggaaagagcacctggcagcgatggactatctgcgtcagggtatccacctgcgtggctacgcacagaaagatccgaagcaggaatacaaacgtgaatcgttctccatgtttgcagcgatgctggagtcgttgaaatatgaagttatcagtacgctgagcaaagttcaggtacgtatgcctgaagaggttgaggagctggaacaacagcgtcgtatggaagccgagcgtttagcgcaaatgcagcagcttagccatcaggatgacgactctgcagccgcagctgcactggcggcgcaaaccggagagcgcaaagtaggacgtaacgatccttgcccgtgcggttctggtaaaaaatacaagcagtgccatggccgcctgcaataaaagctaactgttgaagtaaaaggtgcaggattctgcgccttttttataggtttaagacaa

SEQ ID NO: 47 - DNA, 575 bp, Artificial Sequence
  DCW47b
gctaactgttgaagtaaaaggtgcaggattctgcgccttttttataggtttaagacaatgaaaaagctgcaaattgcggtaggtattattcgcaacgagaacaatgaaatctttataacgcgtcgcgcagcagatgcgcacatggcgaataaactggagtttcccggcggtaaaattgaaatgggtgaaacgccggaacaggcggtggtgcgtgaacttcaggaagaagtcgggattaccccccaacatttttcgctatttgaaaaactggaatatgaattcccggacaggcatataacactgtggttttggctggtcgaacgctgggaaggggagccgtggggtaaagaagggcaacccggtgagtggatgtcgctggtcggtcttaatgccgatgattttccgccagccaatgaaccggtaattgcgaagcttaaacgtctgtaggtcagataaggcgttttcgccgcatccgacattcgcacacgatgcctgatgcgacgctggcgcgtcttatcaggcctaaagggatttctaactcattgataaatttgtttttgtaggtcggataaggc

SEQ ID NO: 48 - DNA, 559 bp, Artificial Sequence
  DCW48b
tttgtttttgtaggtcggataaggcgttcacgccgcatccgacatttgcacaagatgcctgatgcgacgctgtccgcgtcttatcaggcctacgtgcggcatcagacaaatgtcactgctttggttcttcgctccagtcatcgctttcggaaagatcgccactgctggggattcgtttttcttcagcagcccattctccgaggtcgatcagctgacaacgtttggagcaaaatggccgaaacgggctgatttcaccccacaccaccgttttcccgcaggttgggcaattcaccgtaatagtttctgacatttttactccttagcaacaggccagttcgaaatccagacgttccggtacctgtccgttttcagtgtccagcggcataaaacgaatggcaaaacggctcttatgtccggaaatttgcggataaagctgtgaatcgagcgacagattcaggcgcagcaagtcggcatcgccaccgttatcctgataaaaaccattcaggctggtttgtttacggaagggggccgactggcgaattaaatccagcaccatggt

SEQ ID NO: 49 - DNA, 558 bp, Artificial Sequence
  DCW49
tttgtttacggaagggggccgactggcgaattaaatccagcaccatggtaagtgcctgggtgagcgggttcaggctggcaatccaggtttctacctggctgtcgcgctgcgcctggggtagatgcagccaaatgtgcaatgtaggtaaatcaaagctgcaacagccgcctgggatgctcagtcgctgacgcaccagagcaatcaaacgatcttcacgcagaaattgcccgatacgcggcgcggaaattaatacgctccccgccgcttttaactgctgaattaatgcttcaatacggctctggtccacgccaggcacgccaatccaggtctggagtttacgttgctgccggtcaagttctttcaacagctcagtgcggacttcgccgcgctcgaaaacatccagtaattcactgacattacggaagaaatgcagcgcgccagcgtggtcaacgatgggtaaattaacggtgagttgctgaatcaaaaactcaatgcgcagccatgtacgcattttttcatttagtggatgttcaaaaaggacctgggtctgcattacgg

SEQ ID NO: 50 - DNA, 1298 bp, Artificial Sequence
  Cm-oriC (DCW20)
gccgcgcgttatggatacgcgtatgacaccgcctggcctggataaattacccgaagccgtgtcggcttgagaaagacctgagtatgttgtaactaaaggtgcgcataatgtatattatgttaaatggatcctgggtattaaaaagaagatctatttatttagagatctgttctattgtgatctcttattaggatcgcactgccctgtggataacaaggatccggcttttaagatcaacaacctggaaaggatcattaactgtgaatgatcggtgatcctggaccgtataagctgggatcagaatgaggggttatacacaactcaaaaactgaacaacagttgttctttggataactaccggttgatccaagcttcctgacagagttatccacagtagatcgcacgatctgtataacttcgtatagcatacattatacgaagttatctttagttacaacatactccattcttctgccggatcttcttacgccccgccctgccactcatcgcagtactgttgtaattcattaagcattctgccgacatggaagccatcacagacggcatgatgaacctgaatcgccagcggcatcagcaccttgtcgccttgcgtataatatttgcccatggtgaaaacgggggcgaagaagttgtccatattggccacgtttaaatcaaaactggtgaaactcacccagggattggctgagacgaaaaacatattctcaataaaccctttagggaaataggccaggttttcaccgtaacacgccacatcttgcgaatatatgtgtagaaactgccggaaatcgtcgtggtattcactccagagcgatgaaaacgtttcagtttgctcatggaaaacggtgtaacaagggtgaacactatcccatatcaccagctcaccgtctttcattgccatacggaattccggatgagcattcatcaggcgggcaagaatgtgaataaaggccggataaaacttgtgcttatttttctttacggtctttaaaaaggccgtaatatccagctgaacggtctggttataggtacattgagcaactgactgaaatgcctcaaaatgttctttacgatgccattgggatatatcaacggtggtatatccagtgatttttttctccattttagcttccttagctcctgaaaatctcgataactcaaaaaatacgcccggtagtgatcttatttcattatggtgaaagttggaacctcttacgttctaaaaccgtgactgcggatatcccgattgtgggggatgctcgccaggtcctcgaaca

SEQ ID NO: 51 - DNA, 1298 bp, Artificial Sequence
  Cm-oriC (DCW25)
gtctgcgtggaaaaggtataaaagcactgatagctgccccgctgcgtatcttcaacgcctgtcggcttgagaaagacctgagtatgttgtaactaaaggtgcgcataatgtatattatgttaaatggatcctgggtattaaaaagaagatctatttatttagagatctgttctattgtgatctcttattaggatcgcactgccctgtggataacaaggatccggcttttaagatcaacaacctggaaaggatcattaactgtgaatgatcggtgatcctggaccgtataagctgggatcagaatgaggggttatacacaactcaaaaactgaacaacagttgttctttggataactaccggttgatccaagcttcctgacagagttatccacagtagatcgcacgatctgtataacttcgtatagcatacattatacgaagttatctttagttacaacatactccattcttctgccggatcttcttacgccccgccctgccactcatcgcagtactgttgtaattcattaagcattctgccgacatggaagccatcacagacggcatgatgaacctgaatcgccagcggcatcagcaccttgtcgccttgcgtataatatttgcccatggtgaaaacgggggcgaagaagttgtccatattggccacgtttaaatcaaaactggtgaaactcacccagggattggctgagacgaaaaacatattctcaataaaccctttagggaaataggccaggttttcaccgtaacacgccacatcttgcgaatatatgtgtagaaactgccggaaatcgtcgtggtattcactccagagcgatgaaaacgtttcagtttgctcatggaaaacggtgtaacaagggtgaacactatcccatatcaccagctcaccgtctttcattgccatacggaattccggatgagcattcatcaggcgggcaagaatgtgaataaaggccggataaaacttgtgcttatttttctttacggtctttaaaaaggccgtaatatccagctgaacggtctggttataggtacattgagcaactgactgaaatgcctcaaaatgttctttacgatgccattgggatatatcaacggtggtatatccagtgatttttttctccattttagcttccttagctcctgaaaatctcgataactcaaaaaatacgcccggtagtgatcttatttcattatggtgaaagttggaacctcttacgttctaaaaccgtgactgcggatatcccgattgtgggggatgctcgccaggtcctcgaaca

SEQ ID NO: 52 - DNA, 1509 bp, Artificial Sequence
  Km-oriC (DCW25)
gtctgcgtggaaaaggtataaaagcactgatagctgccccgctgcgtatcttcaacgcctgtcggcttgagaaagacctgagtatgttgtaactaaaggtgcgcataatgtatattatgttaaatggatcctgggtattaaaaagaagatctatttatttagagatctgttctattgtgatctcttattaggatcgcactgccctgtggataacaaggatccggcttttaagatcaacaacctggaaaggatcattaactgtgaatgatcggtgatcctggaccgtataagctgggatcagaatgaggggttatacacaactcaaaaactgaacaacagttgttctttggataactaccggttgatccaagcttcctgacagagttatccacagtagatcgcacgatctgtataacttcgtatagcatacattatacgaagttatctttagttacaacatactccattcttctgccggatcttcgggaaagccacgttgtgtctcaaaatctctgatgttacattgcacaagataaaaatatatcatcatgaacaataaaactgtctgcttacataaacagtaatacaaggggtgttatgagccatattcaacgggaaacgtcttgctcgaggccgcgattaaattccaacatggatgctgatttatatgggtataaatgggctcgcgataatgtcgggcaatcaggtgcgacaatctatcgattgtatgggaagcccgatgcgccagagttgtttctgaaacatggcaaaggtagcgttgccaatgatgttacagatgagatggtcagactaaactggctgacggaatttatgcctcttccgaccatcaagcattttatccgtactcctgatgatgcatggttactcaccactgcgatccccgggaaaacagcattccaggtattagaagaatatcctgattcaggtgaaaatattgttgatgcgctggcagtgttcctgcgccggttgcattcgattcctgtttgtaattgtccttttaacagcgatcgcgtatttcgtctcgctcaggcgcaatcacgaatgaataacggtttggttgatgcgagtgattttgatgacgagcgtaatggctggcctgttgaacaagtctggaaagaaatgcataagcttttgccattctcaccggattcagtcgtcactcatggtgatttctcacttgataaccttatttttgacgaggggaaattaataggttgtattgatgttggacgagtcggaatcgcagaccgataccaggatcttgccatcctatggaactgcctcggtgagttttctccttcattacagaaacggctttttcaaaaatatggtattgataatcctgatatgaataaattgcagtttcatttgatgctcgatgagtttttctaatcagaattggttaattggttgtaacactggcagagcttctaaaaccgtgactgcggatatcccgattgtgggggatgctcgccaggtcctcgaaca

SEQ ID NO: 53 - DNA, 1509 bp, Artificial Sequence
  Km-oriC (DCW35)
agtcacatcttaacggtgaagctgaagtagaaaaacgtgttacagcatcagttggctcgtgtcggcttgagaaagacctgagtatgttgtaactaaaggtgcgcataatgtatattatgttaaatggatcctgggtattaaaaagaagatctatttatttagagatctgttctattgtgatctcttattaggatcgcactgccctgtggataacaaggatccggcttttaagatcaacaacctggaaaggatcattaactgtgaatgatcggtgatcctggaccgtataagctgggatcagaatgaggggttatacacaactcaaaaactgaacaacagttgttctttggataactaccggttgatccaagcttcctgacagagttatccacagtagatcgcacgatctgtataacttcgtatagcatacattatacgaagttatctttagttacaacatactccattcttctgccggatcttcgggaaagccacgttgtgtctcaaaatctctgatgttacattgcacaagataaaaatatatcatcatgaacaataaaactgtctgcttacataaacagtaatacaaggggtgttatgagccatattcaacgggaaacgtcttgctcgaggccgcgattaaattccaacatggatgctgatttatatgggtataaatgggctcgcgataatgtcgggcaatcaggtgcgacaatctatcgattgtatgggaagcccgatgcgccagagttgtttctgaaacatggcaaaggtagcgttgccaatgatgttacagatgagatggtcagactaaactggctgacggaatttatgcctcttccgaccatcaagcattttatccgtactcctgatgatgcatggttactcaccactgcgatccccgggaaaacagcattccaggtattagaagaatatcctgattcaggtgaaaatattgttgatgcgctggcagtgttcctgcgccggttgcattcgattcctgtttgtaattgtccttttaacagcgatcgcgtatttcgtctcgctcaggcgcaatcacgaatgaataacggtttggttgatgcgagtgattttgatgacgagcgtaatggctggcctgttgaacaagtctggaaagaaatgcataagcttttgccattctcaccggattcagtcgtcactcatggtgatttctcacttgataaccttatttttgacgaggggaaattaataggttgtattgatgttggacgagtcggaatcgcagaccgataccaggatcttgccatcctatggaactgcctcggtgagttttctccttcattacagaaacggctttttcaaaaatatggtattgataatcctgatatgaataaattgcagtttcatttgatgctcgatgagtttttctaatcagaattggttaattggttgtaacactggcagagcttctaaaaccgtgactgcggatatcccgattgtgggggatgctcgccaggtcctcgaaca

SEQ ID NO: 54 - DNA, 3100 bp, Artificial Sequence
  Lter1
aatagaaaactgccagtgcgcaacctgtaccggttcatgcaatttaaacagacaaatcggtctgccattgatcatattttctgacaaaagctcgccacactgttcaaacccgcgacgccagcgttcagcagtggcgttttgatggcaacgcaaagaaatgtgatcggcagtcagcggagtgatattcaaccccagacggcgggaaagttcatctaatgcgtggataaatcgcggtaaatccgatgcaatatcctgcagctcgtcgatagattgccagttcgccataatcactcttcgtctttcagtaaaagcgttaatttaccctgttgccctgtgccaaccaaccgctgatttcacgccgcttctgatgcaatagtgaaaacggcaatacgccacgcgcacgttgctgacgaaaacagccatttgcagtatactcccgccctaatttctttaactggtgcgggcaatttttgctcgcttcatcaatgtaaggtattccggtgaatattcaggctcttctctcagaaaaagtccgtcaggccatgattgcggcaggcgcgcctgcggattgcgaaccgcaggttcgtcagtcagcaaaagttcagttcggcgactatcaggctaacggcatgatggcagttgctaaaaaactgggtatggcaccgcgacaattagcagagcaggtgctgactcatctggatcttaacggtatcgccagcaaagttgagatcgccggtccaggctttatcaacattttccttgatccggcattcctggctgaacatgttcagcaggcgctggcgtccgatcgtctcggtgttgctacgccagaaaaacagaccattgtggttgactactctgcgccaaacgtggcgaaagagatgcatgtcggtcacctgcgctctaccattattggtgacgcagcagtgcgtactctggagttcctcggtcacaaagtgattcgcgcaaaccacgtcggcgactggggcactcagttcggtatgctgattgcatggctggaaaagcagcagcaggaaaacgccggtgaaatggagctggctgaccttgaaggtttctaccgcgatgcgaaaaagcattacgatgaagatgaagagttcgccgagcgcgcacgtaactacgtggtaaaactgcaaagcggtgacgaatatttccgcgagatgtggcgcaaactggtcgacatcaccatgacgcagaaccagatcacctacgatcgtctcaacgtgacgctgacccgtgatgacgtgatgggcgaaagcctctacaacccgatgctgccaggaattgtggcggatctcaaagccaaaggtctggcagtagaaagcgaaggggcgaccgtcgtattccttgatgagtttaaaaacaaggaaggcgaaccgatgggcgtgatcattcagaagaaagatggcggctatctctacaccaccactgatatcgcctgtgcgaaatatcgttatgaaacactgcatgccgatcgcgtgctgtattacatcgactcccgtcagcatcaacacctgatgcaggcatgggcgatcgtccgtaaagcaggctatgtaccggaatccgtaccgctggaacaccacatgttcggcatgatgctgggtaaagacggcaaaccgttcaaaacccgcgcgggtggtacagtgaaactggccgatctgctggatgaagccctggaacgtgcacgccgtctggtggcagaaaagaacccggatatgccagccgacgagctggaaaaactggctaacgcggttggtattggtgcggtgaaatatgcggatctctccaaaaaccgcaccacggactacatcttcgactgggacaacatgctggcgtttgagggtaataccgcgccatacatgcagtatgcatacacgcgtgtattgtccgtgttccgtaaagcagaaattgacgaagagcaactggctgcagctccggttatcatccgtgaagatcgtgaagcgcaactggcagctcgcctgctgcagtttgaagaaaccctcaccgtggttgcccgtgaaggcacgccgcatgtaatgtgtgcttacctgtacgatctggccggtctgttctctggcttctacgagcactgcccgatcctcagcgcagaaaacgaagaagtgcgtaacagccgtctaaaactggcacaactgacggcgaagacgctgaagctgggtctggatacgctgggtattgagactgtagagcgtatgtaatcgatttttcgtgagagtgaagcctgatcatgacctggcaaagcagaaagcacaatcctcaggcgggttaccgggtcaaaggtggtcgtccggcgctggtggtggtgtttctctgtggtattgctgtgattggcgtgcaatttttgattgcggcagggttgttaccagaagtggggtgatcagatagcctcaaattccttattgggtgccagaattaacgctgacacccaatttggcctcttaatgcaggcagcactgcttaaatttcttaccactaccgcacgggcaaggatcgttacgccccggtttctcttctgctttgatcggttgctgaacagctttttcctgcggatgcgccatccagtacgcatgtagatcaagcgccgccagtcgaatggcatctacgctctcttcaaacgcttctggcgacatcttttctacccgctcgaagttttcctcagtaccgtgcagcgcaatcgcctccagcgctggttttaacgaatcgggcaacgttgaccagtcagaaagtgccacgccccgcatatagccaaagcaccactcctcaacaatcgtcagctcgctgccatcaacttctcgcaagccgaataacggctcaaactgctccgggaattcgttcagacgctctgcggtatcggccatatgttgaaaagccagattcataaagcgcgtcatctctttctctgacgcccagcgcggcacatagtcagccccaccccacacggcaaccagccactgttccggttcaatctcttgcggagaactcaacaccgccgtcaataaaccgtccagctccgccacatcaaggatggcgtggtcagtgttgtatttggtcagaatatcgtcca

SEQ ID NO: 55 - DNA, 3100 bp, Artificial Sequence
  Lter2
ccagctccgccacatcaaggatggcgtggtcagtgttgtatttggtcagaatatcgtccagccattccaactcactttcgtttaacggtcccgttttcatacgcttttccttgtggatctcaactcgccagcacctatcttacatgccggtccgtatcagagatactttttgagtggctttgctggtgattaaaaattaaggagggtgtaacgacaagttgcaggcacaaaaaaaccacccgaaggtggtttcacgacactgcttattgctttgattttattcttatctttcccatggtacccggagcgggacttgaacccgcacagcgcgaacgccgagggattttaaatcccttgtgtctaccgattccaccatccgggctcgggaagaaagtggaggcgcgttccggagtcgaaccggactagacggatttgcaatccgctacataaccgctttgttaacgcgccaaattcttcaggcctttcagccagacatccgcttgacgccgatgtcttttaaactggagcgggaaacgagactcgaactcgcgaccccgaccttggcaaggtcgtgctctaccaactgagctattcccgcattcatcaagcaatcagttaatcacttgattttattatcgtctggcaatcagtgccgccgttcgatgcgttgcattctacttacctggcgcgatgagtcaacgatatttttcaccacttttgatcgtttgctgaaaattacgccgaaacgatcactgatcaagcaaatctgcacgcgcagcgctcaaatattgcaacattgaccacagagtcagtaccgcagccacaaagaaaagtgcaataccggcgtactcaacccaaatgttcggacgccacagcagccatgccaacgccaccatctgggcagtggttttcactttcccaatccaggagacggccacgctactgcgtttacccaactccgccatccattcgcgtagcgcagaaataataatttcacgggcgatcatcgttgccgccggtaatgtcacccaccagctgtgataatgctcggttaccagcaccatggcgatagccacgagaactttatctgccacagggtcaaggaaagcaccaaaccgggtactctggttccagcggcgtgccagaaaaccatcgaaccagtcagtcaccgccgcgacgcagaaaatgagcgcggcggcaaacggcgaccaggtgacaggcagataaaagaccaatacaaagaatgggataaggatgacacggaacagtgtaagcaacgtagggatattaaattgcataatgacgggtaactatctgttgtcagtaagattacccctatgttgctacagagacatcaatgtttcaacgaccagaagatcttttctgccagaccttgcgaaatacccggcacttttaatcgtgggctgtttgcttccttgggcggatacgagttttattatcgtcttaatgatttccacatattaaaagcaagtatgctttcaaaacacaattataaaaaatcccgccaacaatataagtttttataaaattaaatataagattatggctttagaatatttttatttctaatagacgagatttttcctgttatgatataatatgctgaattaacacatgttaacgatttaccagtaatgtaaataaattttcgaggagatcattccagtgggacgtaaatgggccaatattgttgctaaaaaaacggctaaagacggtgcaacgtctaaaatttatgcaaaattcggtgtagaaatctatgctgctgctaaacaaggtgaacccgatccagaattaaacacatctttaaaattcgttattgaacgtgcaaagcaggcacaagttccaaagcacgttattgataaagcaattgataaagccaaaggcggcggagatgaaacgttcgtgcagggacgttatgaaggctttggtcctaatggctcaatgattatcgccgagacattgacttcaaatgttaaccgtacgattgctaacgttcgcacaattttcaataaaaaaggcggcaatatcggagcggcaggttctgtcagctatatgtttgacaatacgggtgtgattgtatttaaagggacagaccctgaccatatttttgaaattttacttgaagctgaagttgatgttcgtgatgtgactgaagaagaaggtaacattgttatttatactgaacctactgaccttcataaaggaatcgcggctctaaaagcagctggaatcactgagttctcaacaacagaattagaaatgattgctcaatctgaagttgagctttccccagaagatttagaaatctttgaagggcttgttgatgcccttgaagatgacgacgatgtacaaaaagtttatcataacgtcgcaaatctctaattatcttttaaagaaatctgtctttacggcagatttctttaatctcatataattcttataaaaaatataatattcaactcgtcatattgattatacccccccgttcccagagaaataatatttattaaaattccagttcttctttttctgattacagaaggcaaagtggcaattacgcatagtttcccgataaagacgcgatagcgacatcccgcataaggcatttttctctttatctttgtacggtacttcatggaacagagtttttgaccttgcgaatcgtgatgtctgttggggagggacaatttgctcactgaagcgtgagactcgattaagcgcacgaaacacagaaatcaaaaaacccggtcacttttttacaaggtaaccgggtaaaaataatttttattttttaactgttttgagactcatagagatgtctcaaaactaaaatttggctcctctgactggactcgaaccagtgacatacggattaacagtccgccgttctaccgactgaactacagaggaatcgtgagaacgaggcgaatattagcgatgcccacccacaatgtcaaagcctgttttttaaatttgaaatcgtttgctgaaataatctgcattttgtcgtttattccgacacaactggctttttttcacacttttgcggctcgggtcgagggtatttccatagccaacg

SEQ ID NO: 56 - DNA, 3100 bp, Artificial Sequence
  Lter3
cacaactggctttttttcacacttttgcggctcgggtcgagggtatttccatagccaacgtccagtaaccattcgccagtaaaacagcacggcccgcacagcccagtcggcaaacattcccatccagacaccaaccacaccccagccaagcatgattcccagcacataaccgactacaacccgacaaccccacatgctcaacatcgaaacccacatggcgtaacgggcatcacgagcacctttaaatccagcgggtagcacccatgaggcggaccaaataggcataaataaagcatttagccaaatcagaatcacaacgacatgtttaacctgtggatcctgggtgtaaaacgatgccataaccccggcaaagggagccgttagccaggcgatggccgttaatccaagagtggaaagccagaacacatgccgcaactgaatctctgcttgcgctatctgccctacccccaaccttcggcctgtaatgatcgtagaagcagagccgagcgcacttccgggtaagttgataagagccgcaattgaaaacgcgataaaatttccggcaataacactggtccccatcccggcaacgaacatttgggttaataaccgaccactggtaaataacactgattcgacactcgcgggaataccaatccccatgacttcccagataatgctaaaattcagcggtttaaaatagctctttaacgaaatccttagcgcaggattaaaaccaatcgccagcacccacaaaattgcaactgcgccaatataacgagaaatggttaaacccagccctgccccgacaaatcccagtcccggccaggagaaaaggccgtaaatcaatatgccgctaataataatattaagaatattcaggctaccgttaatcaatagcggtattttcgtattccctgcaccacgaagtgccccgctaccaataagagtgatggcagctgctggataactgagtaccgtcagctccagataagtcaacgccagtgctttaacttctgtcgtggcatcacccgcgacgaaatcaataatttgttcgccaaaatgatgaataagcgttgccaacagtacggcaaacaacgtcatgatcaccaatgactgccgcgtcgccaccctcgctcgtcgtcgatcccgcttaccgagactaaatgccacaacgacagtagtaccaagatcgatagcagcaaaaaaagccataatgaccatattgaagctgtccgccaatcccacgccggccatcgcatcttttcccagccagctgaccagaaaagtgctcagaacccccatcaacaggacacaggcattctccatgaagataggaacagcaagcggggttatctcgcgccagaacaacactttgtagctcttgcgtttagcgtgccagcgagtgccgtgaacaacctggcgtaaagcagaggagatattcaaagccgaccttaattgcagaaagtgaaaccacatttcaaataatgagggagaatcagcaaagctgcaaagattttcgccaacaaattgtctgcaaatgcaacaaactgttgatagaaacggcaaacagttggggaatttaaaaatcgggtttgacaaaagatttttcgccgttaagatgtgcctcaacaacgattcctctgtagttcagtcggtagaacggcggactgttaatccgtatgtcactggttcgagtccagtcagaggagccaaattcctgaaaagcccgcttttatagcgggatttttgctatatctgataatcaatttcctcttcactgctttccatcacctgccgcttgatatcctcaactgacagtcctgcattacaaagttccagaaagcgccagacatagttacgctgaagttgtcctcgcttcagtcccaaccagacagtattagcatcaaaaagatgccgcgtatccaggcggattaaattctcttcctcttgttcgccactggattgctcggcaactaatccgatcccaagcccaagagcaacataggttttaatgacatcagaatcctgcgcacttaatacaatatctgccagcaaacctttgcgggcaaatgcgtcatcaatacgtgagcgccccgtaatcccctgtcggtaagtgattaacggccacttcgctattgattccagcgtcaatggtgaaatttgcgtcaagggatgatcgtgtggaacaagcaaactatggtgccaacgaaaccacgggaaggcgacgagctgcgggtcattactcaaacgctcgctggcgataccaatatcagcttcgccattttgcaacaatgtcgcaatttcctgtggcgtcccctggattagctcgagccgaacctccgggaaaagttcgcgaaaagctttaatgacctctggcaagctataacgtgcctgagtatgcgtcgttgcaatagtgagaacgccagacgtatcgttggtaaacaggtctgcaagccgacgaacattactggcttcattcagaatacgttctgcaatgaccagtaatgctttgcccggttcagtcatgcccagcagtcgcttacctcgtcgaacaaatatttcgatgccaagttcatcctccagttcccgaatatgacggctgacgcctgactgtgaggtaaaaagcatattcgcaacctctgtcaggttgtaatcctgacgtgcagcctcgcggattatctttagttgttggaaattcacggtaaactccgggcagttcagatttcccgttattgttaaagtctaatgcccggcataacaaataataaaaacccgcatcttattccatcccgatataacacttagctcaccaattgccactgccttttttccatcactggagaactaatcactgacattaacaactctttcactgcctgtgcctgtggcgataagttcgctctggcgggtaaatttaatgacaaagagagactcatggaaggagtggtaatgcgtgacatccacccatttactgcgccacataacgaacgcgcggccgattcgggtaatactgcaacgcccatgccgctggcaatcgctgcggtaagcgtggcaatagactcaatttcaccaataacttttgccgtgagtcgccgta

SEQ ID NO: 57 - DNA, 3100 bp, Artificial Sequence
  Lter4
ctgcggtaagcgtggcaatagactcaatttcaccaataacttttgccgtgagtcgccgtagggaaaaagcctcatcaacacgaagtctaatagcactgtaatcactggggagaaagaggttcatttgcgcaatagcattcacatcaacgctttgccccgggcaatcttgagttcctaccagaaaaagatcttctttcagcaaagcctgactggatacaccagccacaggggaatgctcataaatcaccgccatatcgagttggtgatttatcaatttttcgttaagcactgcaccactattttcatgaagatagataacgatctccggaaattcagcgcgaaccgcctgtaataagggcatggtgatggatgacgcagcggttcctggtgcaaagccaatcgagacttgccccgataatgcctgaccaacgttatgcaccgccagttgggcctgttcacactgacgtaaaatggcccgcgcatgggtatagagaatttttccggcgtctgttggtgtaacgccccgctttgtacggatcaaaagttgttgatttaactcaccttccagtgtggcaacctgctggctgagcgctggttgtgcgatatgcaatacttcagcagcctgggtcaggctaccaatatctacaatttttacgaagtatttcaggcgtctgaagttcatgttgcctccggtttttaagaatcggcccaagtgccgccattacttacaaccagattgcaagatgcttgccagttttattttggtgttgatgtacaagctaaccaactgtcaaataagagattatgatagattcgtcatttgctcctttaatcagctgtcgcgttcccctgccctataaaaggagggtatgcaccacgatggttcattacccaataagattgaaagctcaccactttgttgaaattgacagcaaacaaacaaaaaaatgcatttcaccctttgacatcaccatgcactgccattaatatgcgccccgttcacacgattcctctgtagttcagtcggtagaacggcggactgttaatccgtatgtcactggttcgagtccagtcagaggagccaaattcaaaaaagcctgctttctagcaggctttttgctttctaattaccaacgctcttaaaacatctgtcttgaaccagaactaatttgcacaggcattcccgatcgacgttgcaacgcagcatttgcgcgatttacatcaacttcttgcccgttgataaacgcccgcaaagatggggttaccggcaatggcacttttcggtcagactcatattctgcacgattgcgcgacaatggctcatgaacttccagccagttcgagccatctggttcagtggtgtattttactggctggtcgataatttgcacacgcgtcccaacaggaacattatcaaacagatatttgatatcgtcattgcgcagacgaatacagccctgacttacccggagcccaataccaaaattggcattggtaccatggatggcatacaacctgccaatataaatcgcgtacagccccatgggattatcggggcccgcaggaacaaatgcgggcaaactctcccctcgtttcgcatattcgcgccgagtgttcggcgttggcgtccaggttggagcttcttgtttacgttcaacggtagtcacccagttacgcggggtttctcgcccagcctggccgataccaataggaaagacttccacagtattactgtctggtgggtagtaataaagacgcatctcagcgacgttaacaacaatccctttacgaacagtgtcgggcaaaatcagttgctgcggaatggtgagttgcgagccagacttcggcaaaaaaacatcagcgcccgggttcgcttccagcatgttacttaacccttgcccgtattgtgcggcaaaagtctccagcggctgggtattgtgatcaggaacagttacagtaaacgactgccccactaaacggctaccctctggaggtaatggataagttaccgccaggctagtatggctggcaaaaagcagagcaaatgagcaaagaatatttacacgacgcatcatgtccctttcctatgtcgcgaaagctatccgttaagtatagcttttatcagacttttcgtttttaactgttcaaatcagaagtcgtattccccggtagaacattgttcgttcatcccgactccttttttgtatagataaaccatcagctgatagtttacctgaagaatatagagaagtacttacttaacattttcccatttggtactatctaaccccttttcactattaagaagtaatgcctactatgactcaagtcgcgaagaaaattctggtgacgtgcgcactgccgtacgctaacggctcaatccacctcggccatatgctggagcacatccaggctgatgtctgggtccgttaccagcgaatgcgcggccacgaggtcaacttcatctgcgccgacgatgcccacggtacaccgatcatgctgaaagctcagcagcttggtatcaccccggagcagatgattggcgaaatgagtcaggagcatcagactgatttcgcaggctttaacatcagctatgacaactatcactcgacgcacagcgaagagaaccgccagttgtcagaacttatctactctcgcctgaaagaaaacggttttattaaaaaccgcaccatctctcagctgtacgatccggaaaaaggcatgttcctgccggaccgttttgtgaaaggcacctgcccgaaatgtaaatccccggatcaatacggcgataactgcgaagtctgcggcgcgacctacagcccgactgaactgatcgagccgaaatcggtggtttctggcgctacgccggtaatgcgtgattctgaacacttcttctttgatctgccctctttcagcgaaatgttgcaggcatggacccgcagcggtgcgttgcaggagcaggtggcaaataaaatgcaggagtggtttgaatctggcctgcaacagtgggatatctcccgcgacgccccttacttcggttttgaaattccgaacgcgccgggcaaatatttctacgtctggctggacgcaccgattggct

SEQ ID NO: 58 - DNA, 2650 bp, Artificial Sequence
  Lter5
ttgaaattccgaacgcgccgggcaaatatttctacgtctggctggacgcaccgattggctacatgggttctttcaagaatctgtgcgacaagcgcggcgacagcgtaagcttcgatgaatactggaagaaagactccaccgccgagctgtaccacttcatcggtaaagatattgtttacttccacagcctgttctggcctgccatgctggaaggcagcaacttccgcaagccgtccaacctgtttgttcatggctatgtgacggtgaacggcgcaaagatgtccaagtctcgcggcacctttattaaagccagcacctggctgaatcattttgacgcagacagcctgcgttactactacactgcgaaactctcttcgcgcattgatgatatcgatctcaacctggaagatttcgttcagcgtgtgaatgccgatatcgttaacaaagtggttaacctggcctcccgtaatgcgggctttatcaacaagcgttttgacggcgtgctggcaagcgaactggctgacccgcagttgtacaaaaccttcactgatgccgctgaagtgattggtgaagcgtgggaaagccgtgaatttggtaaagccgtgcgcgaaatcatggcgctggctgatctggctaaccgctatgtcgatgaacaggctccgtgggtggtggcgaaacaggaaggccgcgatgccgacctgcaggcaatttgctcaatgggcatcaacctgttccgcgtgctgatgacttacctgaagccggtactgccgaaactgaccgagcgtgcagaagcattcctcaatacggaactgacctgggatggtatccagcaaccgctgctgggccacaaagtgaatccgttcaaggcgctgtataaccgcatcgatatgaggcaggttgaagcactggtggaagcctctaaagaagaagtaaaagccgctgccgcgccggtaactggcccgctggcagatgatccgattcaggaaaccatcacctttgacgacttcgctaaagttgacctgcgcgtggcgctgattgaaaacgcagagtttgttgaaggttctgacaaactgctgcgcctgacgctggatctcggcggtgaaaaacgcaatgtcttctccggtattcgttctgcttacccggatccgcaggcactgattggtcgtcacaccattatggtggctaacctggcaccacgtaaaatgcgcttcggtatctctgaaggcatggtgatggctgccggtcctggcgggaaagatattttcctgctaagcccggatgccggtgctaaaccgggtcatcaggtgaaataatcccccttcaaggcgctgcatcgacagcgccttttctttataaattcctaaagttgttttcttgcgattttgtctctctctaacccgcataaaatcgagcgtgacgttgcgctccatggttcctgccttttaatcagttgtgatgacgcacagcgcgcagaaactcgtggcgcgtattctgactggatttgaacaatccaccaagagaggtcgttgtcgtggcactggttgcatcgcggatgccacgcgccttcacgcagtaatgcaccgcgtcgatcgagacagccacgttattggtgcccagcagcgtttgtagcgcaataagaatttgctgcgtcagacgttcctgcacctgcggacgctgggcaaagaactgcacaatgcggttaatttttgacagaccgatcaccgaatctttcgggatataggccaccgtcgctttgccatcgatggtaacaaaatggtgttcacaggtgctggtcagagtgatatcgcgcacggtgaccatttcatcgaccttcattttgttttcaatgagggtgattttcgggaaattggcgtaatccagaccggagaaaatttcatcgacatacattttagcgatgcgatgcggcgtttccatcaaactgtcatcagccaggtcgagattcagcagctgcatgatttcggtcatatgaccagcaataaggcttttgcgcgtttcgttatccatttcatgcacgggcgggcgcagcggtgtttccagtcctcgcgcaactaacgcttcatgaaccagggccgcttctttactgagtgatggcatttatgatttctcctgcaggtgtgacgcctccgccctgcgtgggggcaaagttattaagctgatttacagcctgattattgtgcgtgaggcggcgcacataatccagtattcacagcgataattattgtaattgccgctgcctttcatcagcagatgttaaaacatcgttatgcaaatacggaagtgaaagttactcacagcacattgaataaacggtatgatgaagaaattgcaaacaacacaacaaggagccacgcatggaaatgctcgaagagcaccgctgttttgaaggctggcagcaacgctggcgacacgactccagtaccttaaactgcccgatgacgttcagtatctttctccctccacctcgtgatcacactccgccaccagtgctgtactggctttccggattaacctgcaatgacgagaacttcaccaccaaggcgggtgcccagcgggtagcggcggaactggggattgtactggtgatgccagacaccagcccgcgcggcgaaaaggttgccaacgacgatgg

SEQ ID NO: 59 - DNA, 1298 bp, Artificial Sequence
  Cm-oriC/325k fragment
tattggtaaccagaccggcattttacgtaatgaaccaggcatcctttctcccacaaatatcgtaagaggttccaactttcaccataatgaaataagatcactaccgggcgtattttttgagttatcgagattttcaggagctaaggaagctaaaatggagaaaaaaatcactggatataccaccgttgatatatcccaatggcatcgtaaagaacattttgaggcatttcagtcagttgctcaatgtacctataaccagaccgttcagctggatattacggcctttttaaagaccgtaaagaaaaataagcacaagttttatccggcctttattcacattcttgcccgcctgatgaatgctcatccggaattccgtatggcaatgaaagacggtgagctggtgatatgggatagtgttcacccttgttacaccgttttccatgagcaaactgaaacgttttcatcgctctggagtgaataccacgacgatttccggcagtttctacacatatattcgcaagatgtggcgtgttacggtgaaaacctggcctatttccctaaagggtttattgagaatatgtttttcgtctcagccaatccctgggtgagtttcaccagttttgatttaaacgtggccaatatggacaacttcttcgcccccgttttcaccatgggcaaatattatacgcaaggcgacaaggtgctgatgccgctggcgattcaggttcatcatgccgtctgtgatggcttccatgtcggcagaatgcttaatgaattacaacagtactgcgatgagtggcagggcggggcgtaagaagatccggcagaagaatggagtatgttgtaactaaagataacttcgtataatgtatgctatacgaagttatacagatcgtgcgatctactgtggataactctgtcaggaagcttggatcaaccggtagttatccaaagaacaactgttgttcagtttttgagttgtgtataacccctcattctgatcccagcttatacggtccaggatcaccgatcattcacagttaatgatcctttccaggttgttgatcttaaaagccggatccttgttatccacagggcagtgcgatcctaataagagatcacaatagaacagatctctaaataaatagatcttctttttaatacccaggatccatttaacataatatacattatgcgcacctttagttacaacatactcaggtctttctcaagccgacctagagaataaatttatattgattaaatgaatgtatatttcaaattgattttgtttgtta

SEQ ID NO: 60 - DNA, 1298 bp, Artificial Sequence
  Cm-oriC/220k fragment
caaaactgacataaatctccagagatgtgttcaggagttagaaagattatttcttctattcgtaagaggttccaactttcaccataatgaaataagatcactaccgggcgtattttttgagttatcgagattttcaggagctaaggaagctaaaatggagaaaaaaatcactggatataccaccgttgatatatcccaatggcatcgtaaagaacattttgaggcatttcagtcagttgctcaatgtacctataaccagaccgttcagctggatattacggcctttttaaagaccgtaaagaaaaataagcacaagttttatccggcctttattcacattcttgcccgcctgatgaatgctcatccggaattccgtatggcaatgaaagacggtgagctggtgatatgggatagtgttcacccttgttacaccgttttccatgagcaaactgaaacgttttcatcgctctggagtgaataccacgacgatttccggcagtttctacacatatattcgcaagatgtggcgtgttacggtgaaaacctggcctatttccctaaagggtttattgagaatatgtttttcgtctcagccaatccctgggtgagtttcaccagttttgatttaaacgtggccaatatggacaacttcttcgcccccgttttcaccatgggcaaatattatacgcaaggcgacaaggtgctgatgccgctggcgattcaggttcatcatgccgtctgtgatggcttccatgtcggcagaatgcttaatgaattacaacagtactgcgatgagtggcagggcggggcgtaagaagatccggcagaagaatggagtatgttgtaactaaagataacttcgtataatgtatgctatacgaagttatacagatcgtgcgatctactgtggataactctgtcaggaagcttggatcaaccggtagttatccaaagaacaactgttgttcagtttttgagttgtgtataacccctcattctgatcccagcttatacggtccaggatcaccgatcattcacagttaatgatcctttccaggttgttgatcttaaaagccggatccttgttatccacagggcagtgcgatcctaataagagatcacaatagaacagatctctaaataaatagatcttctttttaatacccaggatccatttaacataatatacattatgcgcacctttagttacaacatactcaggtctttctcaagccgacctagaagcgatcactgctgggttacctgttttaacaacagcggtatgtgggtacgcgcat

SEQ ID NO: 61 - protein, 353 aa, Escherichia coli
  RecA
MAIDENKQKALAAALGQIEKQFGKGSIMRLGEDRSMDVETISTGSLSLDIALGAGGLPMGRIVEIYGPESSGKTTLTLQVIAAAQREGKTCAFIDAEHALDPIYARKLGVDIDNLLCSQPDTGEQALEICDALARSGAVDVIVVDSVAALTPKAEIEGEIGDSHMGLAARMMSQAMRKLAGNLKQSNTLLIFINQIRMKIGVMFGNPETTTGGNALKFYASVRLDIRRIGAVKEGENVVGSETRVKVVKNKIAAPFKQAEFQILYGEGINFYGELVDLGVKEKLIEKAGAWYSYKGEKIGQGKANATAWLKDNPETAKEIEKKVRELLLSNPNSTPDFSVDDSEGVAETNEDF

SEQ ID NO: 62 - DNA, 1509 bp, Artificial Sequence; identical to SEQ ID NO: 53
  Km-oriC (DCW49)

SEQ ID NO: 63 - DNA, 19 bp, Artificial Sequence
  primer
ctatgcggcatcagagcag

SEQ ID NO: 64 - DNA, 19 bp, Artificial Sequence
  primer
gttaagccagccccgacac

SEQ ID NO: 65 - DNA, 500 bp, Artificial Sequence
  primer
cgcgtcagcgggtgttggcgggtgtcggggctggcttaacagtactgcgatgagtggcagggcggggcgtaatttttttaaggcagttattggtgcccttaaacgcctggttgctacgcctgaataagtgataataagcggatgaatggcagaaattcgatgataagctgtcaaacatgagaattggtcgacggcgcgccaaagcttgcatgcctgcagccgcgtaacctggcaaaatcggttacggttgagtaataaatggatgccctgcgtaagcggggcacatttcattacctctttctccgcacccgacatagataataacttcgtatagtatacattatacgaagttatctagtagacttaattaaggatcgatccggcgcgccaatagtcatgccccgcgcccaccggaaggagctgactgggttgaaggctctcaagggcatcggtcgagcttctatgcggcatcagagcagattgtactgagagtgcaccat

SEQ ID NO: 66 - DNA, 60 bp, Artificial Sequence
  primer
tgcgtaagcggggcacatttcattacctctttctccgcacgctctgccagtgttacaacc

SEQ ID NO: 67 - DNA, 60 bp, Artificial Sequence
  primer
taatgtatactatacgaagttattatctatgtcgggtgctaacgcggtatgaaaatggat